European Patent Application EP 4 306 169 A2, published January 17, 2024. Title: MEANS AND METHODS FOR GENERATION OF BREAST STEM CELLS. Applicant: Helmholtz Zentrum Muenchen. Application EP. The sequence listing filed with the application follows.

SEQUENCE LISTING (28 sequences)

SEQ ID NO: 1 - DNA, 20 bp, synthetic construct
  misc_feature 1..20: note = CDH1 primer
  source 1..20: mol_type = other DNA
tgcccagaaaatgaaaaagg

SEQ ID NO: 2 - DNA, 20 bp, synthetic construct
  misc_feature 1..20: note = CDH1 primer
  source 1..20: mol_type = other DNA
gtgtatgtggcaatgcgttc

SEQ ID NO: 3 - DNA, 23 bp, synthetic construct
  misc_feature 1..23: note = ELF5 primer
  source 1..23: mol_type = other DNA
tagggaacaaggaatttttcggg

SEQ ID NO: 4 - DNA, 22 bp, synthetic construct
  misc_feature 1..22: note = ELF5 primer
  source 1..22: mol_type = other DNA
gtacactaaccttcggtcaacc

SEQ ID NO: 5 - DNA, 20 bp, synthetic construct
  misc_feature 1..20: note = FN1 primer
  source 1..20: mol_type = other DNA
cagtgggagacctcgagaag

SEQ ID NO: 6 - DNA, 20 bp, synthetic construct
  misc_feature 1..20: note = FN1 primer
  source 1..20: mol_type = other DNA
tccctcggaacatcagaaac

SEQ ID NO: 7 - DNA, 19 bp, synthetic construct
  misc_feature 1..19: note = GATA3 primer
  source 1..19: mol_type = other DNA
gcccctcattaagcccaag

SEQ ID NO: 8 - DNA, 21 bp, synthetic construct
  misc_feature 1..21: note = GATA3 primer
  source 1..21: mol_type = other DNA
ttgtggtggtctgacagttcg

SEQ ID NO: 9 - DNA, 23 bp, synthetic construct
  misc_feature 1..23: note = KRT8 primer
  source 1..23: mol_type = other DNA
tcctcaggcagctatatgaagag

SEQ ID NO: 10 - DNA, 23 bp, synthetic construct
  misc_feature 1..23: note = KRT8 primer
  source 1..23: mol_type = other DNA
ggttggcaatatcctcgtactgt

SEQ ID NO: 11 - DNA, 24 bp, synthetic construct
  misc_feature 1..24: note = RPL32 primer
  source 1..24: mol_type = other DNA
cagggttcgtagaagattcaaggg

SEQ ID NO: 12 - DNA, 25 bp, synthetic construct
  misc_feature 1..25: note = RPL32 primer
  source 1..25: mol_type = other DNA
cttggaggaaacattgtgagcgatc

SEQ ID NO: 13 - DNA, 21 bp, synthetic construct
  misc_feature 1..21: note = MME primer
  source 1..21: mol_type = other DNA
tggatcttgtaagcagcctca

SEQ ID NO: 14 - DNA, 20 bp, synthetic construct
  misc_feature 1..20: note = MME primer
  source 1..20: mol_type = other DNA
gcacaacgtctccaagttgc

SEQ ID NO: 15 - DNA, 20 bp, synthetic construct
  misc_feature 1..20: note = CDH2 primer
  source 1..20: mol_type = other DNA
acagtggccacctacaaagg

SEQ ID NO: 16 - DNA, 20 bp, synthetic construct
  misc_feature 1..20: note = CDH2 primer
  source 1..20: mol_type = other DNA
ccgagatggggttgataatg

SEQ ID NO: 17 - DNA, 21 bp, synthetic construct
  misc_feature 1..21: note = OVOL2 primer
  source 1..21: mol_type = other DNA
acaggcattcgtccctacaaa

SEQ ID NO: 18 - DNA, 21 bp, synthetic construct
  misc_feature 1..21: note = OVOL2 primer
  source 1..21: mol_type = other DNA
cgctgcttataggcatactgc

SEQ ID NO: 19 - DNA, 21 bp, synthetic construct
  misc_feature 1..21: note = TP63 primer
  source 1..21: mol_type = other DNA
agagagagggacttgagttct

SEQ ID NO: 20 - DNA, 21 bp, synthetic construct
  misc_feature 1..21: note = TP63 primer
  source 1..21: mol_type = other DNA
tggtcgatgctgttcaggagc

SEQ ID NO: 21 - DNA, 20 bp, synthetic construct
  misc_feature 1..20: note = SNAI2 primer
  source 1..20: mol_type = other DNA
ggggagaagcctttttcttg

SEQ ID NO: 22 - DNA, 20 bp, synthetic construct
  misc_feature 1..20: note = SNAI2 primer
  source 1..20: mol_type = other DNA
tcctcatgtttgtgcaggag

SEQ ID NO: 23 - DNA, 20 bp, synthetic construct
  misc_feature 1..20: note = VIM primer
  source 1..20: mol_type = other DNA
gagaactttgccgttgaagc

SEQ ID NO: 24 - DNA, 20 bp, synthetic construct
  misc_feature 1..20: note = VIM primer
  source 1..20: mol_type = other DNA
gcttcctgtaggtggcaatc

SEQ ID NO: 25 - DNA, 22 bp, synthetic construct
  misc_feature 1..22: note = ZEB1 primer
  source 1..22: mol_type = other DNA
gcacaagaagagccacaagtag

SEQ ID NO: 26 - DNA, 21 bp, synthetic construct
  misc_feature 1..21: note = ZEB1 primer
  source 1..21: mol_type = other DNA
gcaagacaagttcaagggttc

SEQ ID NO: 27 - DNA, 21 bp, synthetic construct
  misc_feature 1..21: note = TJP1 primer
  source 1..21: mol_type = other DNA
cttaccacactgtgcgtccat

SEQ ID NO: 28 - DNA, 23 bp, synthetic construct
  misc_feature 1..23: note = TJP1 primer
  source 1..23: mol_type = other DNA
aggagtcggatgattttagagca